European Patent Application EP 4 353 837 A2, published April 17, 2024. Title: APTAMERS AS BIOMARKERS. Applicant: NEOVENTURES BIOTECHNOLOGY EUROPE. The sequence listing filed with the application follows.

SEQUENCE LISTING (48 sequences)

SEQ ID NO: 1 - DNA, 86 bp, synthetic construct
  misc_feature 1..86: note = Aptamer library
  misc_feature 1..23: note = /note="Constant region for primer hybridization"
  misc_feature 24..63: note = /note="N can be A, T, C, G, U or any modified nucleotide, preferably N can be A, T, C or G"
  misc_feature 64..86: note = /note="Constant region for primer hybridization"
  source 1..86: mol_type = other DNA
aactacatggtatgtggtgaactnnnnnnnnnnnnnnnnnnnnnnnnnnnnnnnnnnnnnnnngacgtacaatgtaccctatagtg

SEQ ID NO: 2 - DNA, 40 bp, synthetic construct
  misc_feature 1..40: note = Aptamarker
  source 1..40: mol_type = other DNA
cctgcattaccgactagccgccacatagccactcctttca

SEQ ID NO: 3 - DNA, 40 bp, synthetic construct
  misc_feature 1..40: note = Aptamarker
  source 1..40: mol_type = other DNA
gacctcattccaagcccgcaccacagcaccagagccgatg

SEQ ID NO: 4 - DNA, 40 bp, synthetic construct
  misc_feature 1..40: note = Aptamarker
  source 1..40: mol_type = other DNA
ttcgggaccctacgcggcgctcccatccacgcacatccaa

SEQ ID NO: 5 - DNA, 40 bp, synthetic construct
  misc_feature 1..40: note = Aptamarker
  source 1..40: mol_type = other DNA
aaccttttacccttggccattacaccactgccatcctgtc

SEQ ID NO: 6 - DNA, 40 bp, synthetic construct
  misc_feature 1..40: note = Aptamarker
  source 1..40: mol_type = other DNA
ccccggtatccctcgagggcccagccacaacctgctgcca

SEQ ID NO: 7 - DNA, 40 bp, synthetic construct
  misc_feature 1..40: note = Aptamarker
  source 1..40: mol_type = other DNA
cgccgccaatcatagcaacccggccatccacatcctgcga

SEQ ID NO: 8 - DNA, 40 bp, synthetic construct
  misc_feature 1..40: note = Aptamarker
  source 1..40: mol_type = other DNA
gattgaccaggggacccagccatccgaccccacaccagca

SEQ ID NO: 9 - DNA, 40 bp, synthetic construct
  misc_feature 1..40: note = Aptamarker
  source 1..40: mol_type = other DNA
gcccctgattcgactcaaggaccaccgaccatatacctcg

SEQ ID NO: 10 - DNA, 40 bp, synthetic construct
  misc_feature 1..40: note = Aptamarker
  source 1..40: mol_type = other DNA
attcaggtttgacccctcgacacacacaccaccatccaga

SEQ ID NO: 11 - DNA, 40 bp, synthetic construct
  misc_feature 1..40: note = Aptamarker
  source 1..40: mol_type = other DNA
tgaccgttatatatccggctatcgaccacgaccacctgct

SEQ ID NO: 12 - DNA, 40 bp, synthetic construct
  misc_feature 1..40: note = Aptamarker
  source 1..40: mol_type = other DNA
ctagacaggcgcgctacctatttttgccaccacagccacg

SEQ ID NO: 13 - DNA, 40 bp, synthetic construct
  misc_feature 1..40: note = Aptamarker
  source 1..40: mol_type = other DNA
tgtccctgcgtatcctgagaaccgattacacccactacca

SEQ ID NO: 14 - DNA, 40 bp, synthetic construct
  misc_feature 1..40: note = Aptamarker
  source 1..40: mol_type = other DNA
caaccttgactgtcgacaattcaccgcacacccgatcctg

SEQ ID NO: 15 - DNA, 40 bp, synthetic construct
  misc_feature 1..40: note = Aptamarker
  source 1..40: mol_type = other DNA
gaacccacgaattgtcaacccgatccaatcaccacgacca

SEQ ID NO: 16 - DNA, 40 bp, synthetic construct
  misc_feature 1..40: note = Aptamarker
  source 1..40: mol_type = other DNA
tactgatcgatcttcatactccgccacattgaccatcccg

SEQ ID NO: 17 - DNA, 40 bp, synthetic construct
  misc_feature 1..40: note = Aptamarker
  source 1..40: mol_type = other DNA
agcgccaaacagccatatcccgacgataccacataaccga

SEQ ID NO: 18 - DNA, 40 bp, synthetic construct
  misc_feature 1..40: note = Aptamarker
  source 1..40: mol_type = other DNA
cgccgacggttgctctcgacttgcccatcccctgccatga

SEQ ID NO: 19 - DNA, 40 bp, synthetic construct
  misc_feature 1..40: note = Aptamarker
  source 1..40: mol_type = other DNA
gccagtagacgctgaccgccaacccaccgccatccatgag

SEQ ID NO: 20 - DNA, 40 bp, synthetic construct
  misc_feature 1..40: note = Aptamarker
  source 1..40: mol_type = other DNA
tggcactggggctggccgaacaccacccaccctatagcaa

SEQ ID NO: 21 - DNA, 40 bp, synthetic construct
  misc_feature 1..40: note = Aptamarker
  source 1..40: mol_type = other DNA
cgagagacagatatcccttcgcatccactaccaatcgccg

SEQ ID NO: 22 - DNA, 40 bp, synthetic construct
  misc_feature 1..40: note = Aptamarker
  source 1..40: mol_type = other DNA
taggagcagtaccccgatcgaccacaccactctacgggca

SEQ ID NO: 23 - DNA, 40 bp, synthetic construct
  misc_feature 1..40: note = Aptamarker
  source 1..40: mol_type = other DNA
gcccttgaatcgatcccggacttgccacatccacagcaga

SEQ ID NO: 24 - DNA, 40 bp, synthetic construct
  misc_feature 1..40: note = Aptamarker
  source 1..40: mol_type = other DNA
tgccaacagatgactactgcgcacccatcagccacatcca

SEQ ID NO: 25 - DNA, 40 bp, synthetic construct
  misc_feature 1..40: note = Aptamarker
  source 1..40: mol_type = other DNA
atcagaaccttaccggccgtcactttgccaccacaaccga

SEQ ID NO: 26 - DNA, 40 bp, synthetic construct
  misc_feature 1..40: note = Aptamarker
  source 1..40: mol_type = other DNA
gaaccgtcgtctacctcgatcccgcccacagcactaccag

SEQ ID NO: 27 - DNA, 40 bp, synthetic construct
  misc_feature 1..40: note = Aptamarker
  source 1..40: mol_type = other DNA
cactatttcttacaacacgcgcgctttaccaccataccga

SEQ ID NO: 28 - DNA, 40 bp, synthetic construct
  misc_feature 1..40: note = Aptamarker
  source 1..40: mol_type = other DNA
tctgggcccaacagacctcgacccgctgacaccgctacca

SEQ ID NO: 29 - DNA, 40 bp, synthetic construct
  misc_feature 1..40: note = Aptamarker
  source 1..40: mol_type = other DNA
cgccggcatatcgctctaacccgggaccacacccacgact

SEQ ID NO: 30 - DNA, 40 bp, synthetic construct
  misc_feature 1..40: note = Aptamarker
  source 1..40: mol_type = other DNA
tagctcggattgagacgcccacctccacagcccttgaccg

SEQ ID NO: 31 - DNA, 40 bp, synthetic construct
  misc_feature 1..40: note = Aptamarker
  source 1..40: mol_type = other DNA
taggccatcccttcatccacgtagccgccattgaccccga

SEQ ID NO: 32 - DNA, 40 bp, synthetic construct
  misc_feature 1..40: note = Aptamarker
  source 1..40: mol_type = other DNA
tggccatatgttctcccataagctgcaccacaccccttga

SEQ ID NO: 33 - DNA, 40 bp, synthetic construct
  misc_feature 1..40: note = Aptamarker
  source 1..40: mol_type = other DNA
aaggtcgtcgaataacccctcatccaccgccgtaccacaa

SEQ ID NO: 34 - DNA, 40 bp, synthetic construct
  misc_feature 1..40: note = Aptamarker
  source 1..40: mol_type = other DNA
aggccgtcctcgaacatacctaaccacaccccactgaccg

SEQ ID NO: 35 - DNA, 40 bp, synthetic construct
  misc_feature 1..40: note = Aptamarker
  source 1..40: mol_type = other DNA
cagacgccttaacctctacccgagccctgccacgccatgt

SEQ ID NO: 36 - DNA, 40 bp, synthetic construct
  misc_feature 1..40: note = Aptamarker
  source 1..40: mol_type = other DNA
gccccctgctattacacatcgagcattcgcccacacccag

SEQ ID NO: 37 - DNA, 40 bp, synthetic construct
  misc_feature 1..40: note = Aptamarker
  source 1..40: mol_type = other DNA
cccagataacccatcccgacctgagagccccgataccata

SEQ ID NO: 38 - DNA, 40 bp, synthetic construct
  misc_feature 1..40: note = Aptamarker
  source 1..40: mol_type = other DNA
cggctctacctgctctgtccgttccacataacccaaacca

SEQ ID NO: 39 - DNA, 40 bp, synthetic construct
  misc_feature 1..40: note = Aptamarker
  source 1..40: mol_type = other DNA
gtgtgctaccaacagataatgaccactcccaatgagcgcg

SEQ ID NO: 40 - DNA, 40 bp, synthetic construct
  misc_feature 1..40: note = Aptamarker
  source 1..40: mol_type = other DNA
acctctattcccggcgccccaaccacatatccaggacttg

SEQ ID NO: 41 - DNA, 40 bp, synthetic construct
  misc_feature 1..40: note = Aptamarker
  source 1..40: mol_type = other DNA
atcgacttccactctagtctcgaccgcccaccgtaccata

SEQ ID NO: 42 - DNA, 40 bp, synthetic construct
  misc_feature 1..40: note = Aptamarker
  source 1..40: mol_type = other DNA
cagccttttgttaacctgcacccacagtacccgatagaca

SEQ ID NO: 43 - DNA, 40 bp, synthetic construct
  misc_feature 1..40: note = Aptamarker
  source 1..40: mol_type = other DNA
acggacacacgccggctagccacccttaacctatatgtcg

SEQ ID NO: 44 - DNA, 40 bp, synthetic construct
  misc_feature 1..40: note = Aptamarker
  source 1..40: mol_type = other DNA
tgacgctttaatccgccccatagcaccacaccaccaatca

SEQ ID NO: 45 - DNA, 40 bp, synthetic construct
  misc_feature 1..40: note = Aptamarker
  source 1..40: mol_type = other DNA
cagaaaccgctaagcccttgccacagaccagcatgtgccg

SEQ ID NO: 46 - DNA, 40 bp, synthetic construct
  misc_feature 1..40: note = Aptamarker
  source 1..40: mol_type = other DNA
agccggaatgagaacccccgaccaacccatccataccgaa

SEQ ID NO: 47 - DNA, 23 bp, synthetic construct
  misc_feature 1..23: note = 5'-primer recognition sequence region
  source 1..23: mol_type = other DNA
aactacatggtatgtggtgaact

SEQ ID NO: 48 - DNA, 23 bp, synthetic construct
  misc_feature 1..23: note = 3'-primer recognition sequence region
  source 1..23: mol_type = other DNA
gacgtacaatgtaccctatagtg